European Patent Application EP 4 726 038 A1, published April 15, 2026. Title: 表达可调控的工程化RNA分子. Applicant: 仁景（苏州）生物科技有限公司. Application CN. The sequence listing filed with the application follows.

SEQUENCE LISTING (73 sequences)

SEQ ID NO: 1 - DNA, 123 bp, synthetic construct
  source 1..123: mol_type = other DNA
aaaaaaaaaaaaaaaaaaaaaaaaaaaaaaaaaaaaaaaaaaaaaaaaaaaaaaaaaaaagatatcaaaaaaaaaaaaaaaaaaagaaaaaaaaaaaaaaaaaaagaaaaaaaaaaaaaaaaa

SEQ ID NO: 2 - DNA, 20 bp, synthetic construct
  source 1..20: mol_type = other DNA
taatacgactcactataagg

SEQ ID NO: 3 - DNA, 110 bp, synthetic construct
  source 1..110: mol_type = other DNA
gctggagcctcggtggccatgcttcttgccccttgggcctccccccagcccctcctccccttcctgcacccgtacccccgtggtctttgaataaagtctgagtgggcggc

SEQ ID NO: 4 - DNA, 23 bp, synthetic construct
  source 1..23: mol_type = other DNA
tccataaagtaggaaacactaca

SEQ ID NO: 5 - DNA, 133 bp, synthetic construct
  source 1..133: mol_type = other DNA
gctggagcctcggtggccatgcttcttgccccttgggcctccccccagcccctcctccccttcctgcacccgtaccccctccataaagtaggaaacactacagtggtctttgaataaagtctgagtgggcggc

SEQ ID NO: 6 - DNA, 140 bp, synthetic construct
  source 1..140: mol_type = other DNA
aaaaaaaaaaaaaaaaaaaaaaaaaaaaaaaaaaaaaaaaaaaaaaaaaaaaaaaaaaaatccataaagtaggaaacactacaaaaaaaaaaaaaaaaaaaagaaaaaaaaaaaaaaaaaaagaaaaaaaaaaaaaaaaa

SEQ ID NO: 7 - DNA, 146 bp, synthetic construct
  source 1..146: mol_type = other DNA
aaaaaaaaaaaaaaaaaaaaaaaaaaaaaatccataaagtaggaaacactacaaaaaaaaaaaaaaaaaaaaaaaaaaaaaaagatatcaaaaaaaaaaaaaaaaaaagaaaaaaaaaaaaaaaaaaagaaaaaaaaaaaaaaaaa

SEQ ID NO: 8 - DNA, 146 bp, synthetic construct
  source 1..146: mol_type = other DNA
aaaaaaaaaaaaaaaaaaatccataaagtaggaaacactacaaaaaaaaaaaaaaaaaaaaaaaaaaaaaaaaaaaaaaaaaagatatcaaaaaaaaaaaaaaaaaaagaaaaaaaaaaaaaaaaaaagaaaaaaaaaaaaaaaaa

SEQ ID NO: 9 - DNA, 146 bp, synthetic construct
  source 1..146: mol_type = other DNA
aaaaaaaaaaaaaatccataaagtaggaaacactacaaaaaaaaaaaaaaaaaaaaaaaaaaaaaaaaaaaaaaaaaaaaaaagatatcaaaaaaaaaaaaaaaaaaagaaaaaaaaaaaaaaaaaaagaaaaaaaaaaaaaaaaa

SEQ ID NO: 10 - DNA, 146 bp, synthetic construct
  source 1..146: mol_type = other DNA
aaaaaaaaaatccataaagtaggaaacactacaaaaaaaaaaaaaaaaaaaaaaaaaaaaaaaaaaaaaaaaaaaaaaaaaaagatatcaaaaaaaaaaaaaaaaaaagaaaaaaaaaaaaaaaaaaagaaaaaaaaaaaaaaaaa

SEQ ID NO: 11 - DNA, 146 bp, synthetic construct
  source 1..146: mol_type = other DNA
aaaaatccataaagtaggaaacactacaaaaaaaaaaaaaaaaaaaaaaaaaaaaaaaaaaaaaaaaaaaaaaaaaaaaaaaagatatcaaaaaaaaaaaaaaaaaaagaaaaaaaaaaaaaaaaaaagaaaaaaaaaaaaaaaaa

SEQ ID NO: 12 - DNA, 146 bp, synthetic construct
  source 1..146: mol_type = other DNA
aaaatccataaagtaggaaacactacaaaaaaaaaaaaaaaaaaaaaaaaaaaaaaaaaaaaaaaaaaaaaaaaaaaaaaaaagatatcaaaaaaaaaaaaaaaaaaagaaaaaaaaaaaaaaaaaaagaaaaaaaaaaaaaaaaa

SEQ ID NO: 13 - DNA, 146 bp, synthetic construct
  source 1..146: mol_type = other DNA
aaatccataaagtaggaaacactacaaaaaaaaaaaaaaaaaaaaaaaaaaaaaaaaaaaaaaaaaaaaaaaaaaaaaaaaaagatatcaaaaaaaaaaaaaaaaaaagaaaaaaaaaaaaaaaaaaagaaaaaaaaaaaaaaaaa

SEQ ID NO: 14 - DNA, 146 bp, synthetic construct
  source 1..146: mol_type = other DNA
aatccataaagtaggaaacactacaaaaaaaaaaaaaaaaaaaaaaaaaaaaaaaaaaaaaaaaaaaaaaaaaaaaaaaaaaagatatcaaaaaaaaaaaaaaaaaaagaaaaaaaaaaaaaaaaaaagaaaaaaaaaaaaaaaaa

SEQ ID NO: 15 - DNA, 146 bp, synthetic construct
  source 1..146: mol_type = other DNA
atccataaagtaggaaacactacaaaaaaaaaaaaaaaaaaaaaaaaaaaaaaaaaaaaaaaaaaaaaaaaaaaaaaaaaaaagatatcaaaaaaaaaaaaaaaaaaagaaaaaaaaaaaaaaaaaaagaaaaaaaaaaaaaaaaa

SEQ ID NO: 16 - DNA, 146 bp, synthetic construct
  source 1..146: mol_type = other DNA
tccataaagtaggaaacactacaaaaaaaaaaaaaaaaaaaaaaaaaaaaaaaaaaaaaaaaaaaaaaaaaaaaaaaaaaaaagatatcaaaaaaaaaaaaaaaaaaagaaaaaaaaaaaaaaaaaaagaaaaaaaaaaaaaaaaa

SEQ ID NO: 17 - DNA, 22 bp, synthetic construct
  source 1..22: mol_type = other DNA
caaacaccattgtcacactcca

SEQ ID NO: 18 - DNA, 132 bp, synthetic construct
  source 1..132: mol_type = other DNA
gctggagcctcggtggccatgcttcttgccccttgggcctccccccagcccctcctccccttcctgcacccgtaccccccaaacaccattgtcacactccagtggtctttgaataaagtctgagtgggcggc

SEQ ID NO: 19 - DNA, 139 bp, synthetic construct
  source 1..139: mol_type = other DNA
aaaaaaaaaaaaaaaaaaaaaaaaaaaaaaaaaaaaaaaaaaaaaaaaaaaaaaaaaaaacaaacaccattgtcacactccaaaaaaaaaaaaaaaaaaaagaaaaaaaaaaaaaaaaaaagaaaaaaaaaaaaaaaaa

SEQ ID NO: 20 - DNA, 145 bp, synthetic construct
  source 1..145: mol_type = other DNA
aaaaaaaaaaaaaaaaaaaaaaaaaaaaaacaaacaccattgtcacactccaaaaaaaaaaaaaaaaaaaaaaaaaaaaaaagatatcaaaaaaaaaaaaaaaaaaagaaaaaaaaaaaaaaaaaaagaaaaaaaaaaaaaaaaa

SEQ ID NO: 21 - DNA, 145 bp, synthetic construct
  source 1..145: mol_type = other DNA
aaaaaaaaaaaaaaaaaaacaaacaccattgtcacactccaaaaaaaaaaaaaaaaaaaaaaaaaaaaaaaaaaaaaaaaaagatatcaaaaaaaaaaaaaaaaaaagaaaaaaaaaaaaaaaaaaagaaaaaaaaaaaaaaaaa

SEQ ID NO: 22 - DNA, 145 bp, synthetic construct
  source 1..145: mol_type = other DNA
aaaaaaaaaaaaaacaaacaccattgtcacactccaaaaaaaaaaaaaaaaaaaaaaaaaaaaaaaaaaaaaaaaaaaaaaagatatcaaaaaaaaaaaaaaaaaaagaaaaaaaaaaaaaaaaaaagaaaaaaaaaaaaaaaaa

SEQ ID NO: 23 - DNA, 145 bp, synthetic construct
  source 1..145: mol_type = other DNA
aaaaaaaaaacaaacaccattgtcacactccaaaaaaaaaaaaaaaaaaaaaaaaaaaaaaaaaaaaaaaaaaaaaaaaaaagatatcaaaaaaaaaaaaaaaaaaagaaaaaaaaaaaaaaaaaaagaaaaaaaaaaaaaaaaa

SEQ ID NO: 24 - DNA, 145 bp, synthetic construct
  source 1..145: mol_type = other DNA
aaaaacaaacaccattgtcacactccaaaaaaaaaaaaaaaaaaaaaaaaaaaaaaaaaaaaaaaaaaaaaaaaaaaaaaaagatatcaaaaaaaaaaaaaaaaaaagaaaaaaaaaaaaaaaaaaagaaaaaaaaaaaaaaaaa

SEQ ID NO: 25 - DNA, 145 bp, synthetic construct
  source 1..145: mol_type = other DNA
aaaacaaacaccattgtcacactccaaaaaaaaaaaaaaaaaaaaaaaaaaaaaaaaaaaaaaaaaaaaaaaaaaaaaaaaagatatcaaaaaaaaaaaaaaaaaaagaaaaaaaaaaaaaaaaaaagaaaaaaaaaaaaaaaaa

SEQ ID NO: 26 - DNA, 145 bp, synthetic construct
  source 1..145: mol_type = other DNA
aaacaaacaccattgtcacactccaaaaaaaaaaaaaaaaaaaaaaaaaaaaaaaaaaaaaaaaaaaaaaaaaaaaaaaaaagatatcaaaaaaaaaaaaaaaaaaagaaaaaaaaaaaaaaaaaaagaaaaaaaaaaaaaaaaa

SEQ ID NO: 27 - DNA, 145 bp, synthetic construct
  source 1..145: mol_type = other DNA
aacaaacaccattgtcacactccaaaaaaaaaaaaaaaaaaaaaaaaaaaaaaaaaaaaaaaaaaaaaaaaaaaaaaaaaaagatatcaaaaaaaaaaaaaaaaaaagaaaaaaaaaaaaaaaaaaagaaaaaaaaaaaaaaaaa

SEQ ID NO: 28 - DNA, 145 bp, synthetic construct
  source 1..145: mol_type = other DNA
acaaacaccattgtcacactccaaaaaaaaaaaaaaaaaaaaaaaaaaaaaaaaaaaaaaaaaaaaaaaaaaaaaaaaaaaagatatcaaaaaaaaaaaaaaaaaaagaaaaaaaaaaaaaaaaaaagaaaaaaaaaaaaaaaaa

SEQ ID NO: 29 - DNA, 145 bp, synthetic construct
  source 1..145: mol_type = other DNA
caaacaccattgtcacactccaaaaaaaaaaaaaaaaaaaaaaaaaaaaaaaaaaaaaaaaaaaaaaaaaaaaaaaaaaaaagatatcaaaaaaaaaaaaaaaaaaagaaaaaaaaaaaaaaaaaaagaaaaaaaaaaaaaaaaa

SEQ ID NO: 30 - DNA, 168 bp, synthetic construct
  source 1..168: mol_type = other DNA
caaacaccattgtcacactccatccataaagtaggaaacactacaaaaaaaaaaaaaaaaaaaaaaaaaaaaaaaaaaaaaaaaaaaaaaaaaaaaaaaaaaaaagatatcaaaaaaaaaaaaaaaaaaagaaaaaaaaaaaaaaaaaaagaaaaaaaaaaaaaaaaa

SEQ ID NO: 31 - DNA, 168 bp, synthetic construct
  source 1..168: mol_type = other DNA
tccataaagtaggaaacactacacaaacaccattgtcacactccaaaaaaaaaaaaaaaaaaaaaaaaaaaaaaaaaaaaaaaaaaaaaaaaaaaaaaaaaaaaagatatcaaaaaaaaaaaaaaaaaaagaaaaaaaaaaaaaaaaaaagaaaaaaaaaaaaaaaaa

SEQ ID NO: 32 - DNA, 22 bp, synthetic construct
  source 1..22: mol_type = other DNA
cgcattattactcacggtacga

SEQ ID NO: 33 - DNA, 139 bp, synthetic construct
  source 1..139: mol_type = other DNA
aaaaaaaaaaaaaaaaaaaaaaaaaaaaaaaaaaaaaaaaaaaaaaaaaaaaaaaaaaaacgcattattactcacggtacgaaaaaaaaaaaaaaaaaaaagaaaaaaaaaaaaaaaaaaagaaaaaaaaaaaaaaaaa

SEQ ID NO: 34 - DNA, 145 bp, synthetic construct
  source 1..145: mol_type = other DNA
aaaaaaaaaaaaaaaaaaaaaaaaaaaaaacgcattattactcacggtacgaaaaaaaaaaaaaaaaaaaaaaaaaaaaaaagatatcaaaaaaaaaaaaaaaaaaagaaaaaaaaaaaaaaaaaaagaaaaaaaaaaaaaaaaa

SEQ ID NO: 35 - DNA, 145 bp, synthetic construct
  source 1..145: mol_type = other DNA
aaaaaaaaaaaaaaaaaaacgcattattactcacggtacgaaaaaaaaaaaaaaaaaaaaaaaaaaaaaaaaaaaaaaaaaagatatcaaaaaaaaaaaaaaaaaaagaaaaaaaaaaaaaaaaaaagaaaaaaaaaaaaaaaaa

SEQ ID NO: 36 - DNA, 145 bp, synthetic construct
  source 1..145: mol_type = other DNA
aaaaaaaaaaaaaacgcattattactcacggtacgaaaaaaaaaaaaaaaaaaaaaaaaaaaaaaaaaaaaaaaaaaaaaaagatatcaaaaaaaaaaaaaaaaaaagaaaaaaaaaaaaaaaaaaagaaaaaaaaaaaaaaaaa

SEQ ID NO: 37 - DNA, 145 bp, synthetic construct
  source 1..145: mol_type = other DNA
cgcattattactcacggtacgaaaaaaaaaaaaaaaaaaaaaaaaaaaaaaaaaaaaaaaaaaaaaaaaaaaaaaaaaaaaagatatcaaaaaaaaaaaaaaaaaaagaaaaaaaaaaaaaaaaaaagaaaaaaaaaaaaaaaaa

SEQ ID NO: 38 - DNA, 143 bp, synthetic construct
  source 1..143: mol_type = other DNA
tccataaagtaggaaacactacaaaaaaaaaaaaaaaaaaaaaaaaaaaaaaaaaaaaaaaaaaaaaaaaaaaaaaaaaaaaaaaaaaaaaaaaaaaaaaaaaaaaaaaaaaaaaaaaaaaaaaaaaaaaaaaaaaaaaaaaa

SEQ ID NO: 39 - DNA, 142 bp, synthetic construct
  source 1..142: mol_type = other DNA
caaacaccattgtcacactccaaaaaaaaaaaaaaaaaaaaaaaaaaaaaaaaaaaaaaaaaaaaaaaaaaaaaaaaaaaaaaaaaaaaaaaaaaaaaaaaaaaaaaaaaaaaaaaaaaaaaaaaaaaaaaaaaaaaaaaaa

SEQ ID NO: 40 - DNA, 142 bp, synthetic construct
  source 1..142: mol_type = other DNA
cgcattattactcacggtacgaaaaaaaaaaaaaaaaaaaaaaaaaaaaaaaaaaaaaaaaaaaaaaaaaaaaaaaaaaaaaaaaaaaaaaaaaaaaaaaaaaaaaaaaaaaaaaaaaaaaaaaaaaaaaaaaaaaaaaaaa

SEQ ID NO: 41 - DNA, 143 bp, synthetic construct
  source 1..143: mol_type = other DNA
aaaaaaaaaaaaaatccataaagtaggaaacactacaaaaaaaaaaaaaaaaaaaaaaaaaaaaaaaaaaaaaaaaaaaaaaaaaaaaaaaaaaaaaaaaaaaaaaaaaaaaaaaaaaaaaaaaaaaaaaaaaaaaaaaaaaa

SEQ ID NO: 42 - DNA, 142 bp, synthetic construct
  source 1..142: mol_type = other DNA
aaaaaaaaaaaaaacaaacaccattgtcacactccaaaaaaaaaaaaaaaaaaaaaaaaaaaaaaaaaaaaaaaaaaaaaaaaaaaaaaaaaaaaaaaaaaaaaaaaaaaaaaaaaaaaaaaaaaaaaaaaaaaaaaaaaaa

SEQ ID NO: 43 - DNA, 142 bp, synthetic construct
  source 1..142: mol_type = other DNA
aaaaaaaaaaaaaacgcattattactcacggtacgaaaaaaaaaaaaaaaaaaaaaaaaaaaaaaaaaaaaaaaaaaaaaaaaaaaaaaaaaaaaaaaaaaaaaaaaaaaaaaaaaaaaaaaaaaaaaaaaaaaaaaaaaaa

SEQ ID NO: 44 - DNA, 143 bp, synthetic construct
  source 1..143: mol_type = other DNA
aaaaaaaaaaaaaaaaaaatccataaagtaggaaacactacaaaaaaaaaaaaaaaaaaaaaaaaaaaaaaaaaaaaaaaaaaaaaaaaaaaaaaaaaaaaaaaaaaaaaaaaaaaaaaaaaaaaaaaaaaaaaaaaaaaaaa

SEQ ID NO: 45 - DNA, 142 bp, synthetic construct
  source 1..142: mol_type = other DNA
aaaaaaaaaaaaaaaaaaacaaacaccattgtcacactccaaaaaaaaaaaaaaaaaaaaaaaaaaaaaaaaaaaaaaaaaaaaaaaaaaaaaaaaaaaaaaaaaaaaaaaaaaaaaaaaaaaaaaaaaaaaaaaaaaaaaa

SEQ ID NO: 46 - DNA, 142 bp, synthetic construct
  source 1..142: mol_type = other DNA
aaaaaaaaaaaaaaaaaaacgcattattactcacggtacgaaaaaaaaaaaaaaaaaaaaaaaaaaaaaaaaaaaaaaaaaaaaaaaaaaaaaaaaaaaaaaaaaaaaaaaaaaaaaaaaaaaaaaaaaaaaaaaaaaaaaa

SEQ ID NO: 47 - DNA, 143 bp, synthetic construct
  source 1..143: mol_type = other DNA
aaaaaaaaaaaaaaaaaaaaaaaaaaaaaatccataaagtaggaaacactacaaaaaaaaaaaaaaaaaaaaaaaaaaaaaaaaaaaaaaaaaaaaaaaaaaaaaaaaaaaaaaaaaaaaaaaaaaaaaaaaaaaaaaaaaaa

SEQ ID NO: 48 - DNA, 142 bp, synthetic construct
  source 1..142: mol_type = other DNA
aaaaaaaaaaaaaaaaaaaaaaaaaaaaaacaaacaccattgtcacactccaaaaaaaaaaaaaaaaaaaaaaaaaaaaaaaaaaaaaaaaaaaaaaaaaaaaaaaaaaaaaaaaaaaaaaaaaaaaaaaaaaaaaaaaaaa

SEQ ID NO: 49 - DNA, 142 bp, synthetic construct
  source 1..142: mol_type = other DNA
aaaaaaaaaaaaaaaaaaaaaaaaaaaaaacgcattattactcacggtacgaaaaaaaaaaaaaaaaaaaaaaaaaaaaaaaaaaaaaaaaaaaaaaaaaaaaaaaaaaaaaaaaaaaaaaaaaaaaaaaaaaaaaaaaaaa

SEQ ID NO: 50 - DNA, 143 bp, synthetic construct
  source 1..143: mol_type = other DNA
aaaaaaaaaaaaaaaaaaaaaaaaaaaaaaaaaaaaaaaaaaaaaaaaaaaaaaaaaaaatccataaagtaggaaacactacaaaaaaaaaaaaaaaaaaaaaaaaaaaaaaaaaaaaaaaaaaaaaaaaaaaaaaaaaaaaa

SEQ ID NO: 51 - DNA, 142 bp, synthetic construct
  source 1..142: mol_type = other DNA
aaaaaaaaaaaaaaaaaaaaaaaaaaaaaaaaaaaaaaaaaaaaaaaaaaaaaaaaaaaacaaacaccattgtcacactccaaaaaaaaaaaaaaaaaaaaaaaaaaaaaaaaaaaaaaaaaaaaaaaaaaaaaaaaaaaaa

SEQ ID NO: 52 - DNA, 142 bp, synthetic construct
  source 1..142: mol_type = other DNA
aaaaaaaaaaaaaaaaaaaaaaaaaaaaaaaaaaaaaaaaaaaaaaaaaaaaaaaaaaaacgcattattactcacggtacgaaaaaaaaaaaaaaaaaaaaaaaaaaaaaaaaaaaaaaaaaaaaaaaaaaaaaaaaaaaaa

SEQ ID NO: 53 - DNA, 22 bp, synthetic construct
  source 1..22: mol_type = other DNA
acaaagttctgtagtgcactga

SEQ ID NO: 54 - DNA, 190 bp, synthetic construct
  source 1..190: mol_type = other DNA
tccataaagtaggaaacactacacgcattattactcacggtacgaacaaagttctgtagtgcactgaaaaaaaaaaaaaaaaaaaaaaaaaaaaaaaaaaaaaaaaaaaaaaaaaaaaaaaaaaaaagatatcaaaaaaaaaaaaaaaaaaagaaaaaaaaaaaaaaaaaaagaaaaaaaaaaaaaaaaa

SEQ ID NO: 55 - DNA, 190 bp, synthetic construct
  source 1..190: mol_type = other DNA
tccataaagtaggaaacactacaacaaagttctgtagtgcactgacgcattattactcacggtacgaaaaaaaaaaaaaaaaaaaaaaaaaaaaaaaaaaaaaaaaaaaaaaaaaaaaaaaaaaaaagatatcaaaaaaaaaaaaaaaaaaagaaaaaaaaaaaaaaaaaaagaaaaaaaaaaaaaaaaa

SEQ ID NO: 56 - DNA, 190 bp, synthetic construct
  source 1..190: mol_type = other DNA
cgcattattactcacggtacgatccataaagtaggaaacactacaacaaagttctgtagtgcactgaaaaaaaaaaaaaaaaaaaaaaaaaaaaaaaaaaaaaaaaaaaaaaaaaaaaaaaaaaaaagatatcaaaaaaaaaaaaaaaaaaagaaaaaaaaaaaaaaaaaaagaaaaaaaaaaaaaaaaa

SEQ ID NO: 57 - DNA, 190 bp, synthetic construct
  source 1..190: mol_type = other DNA
cgcattattactcacggtacgaacaaagttctgtagtgcactgatccataaagtaggaaacactacaaaaaaaaaaaaaaaaaaaaaaaaaaaaaaaaaaaaaaaaaaaaaaaaaaaaaaaaaaaaagatatcaaaaaaaaaaaaaaaaaaagaaaaaaaaaaaaaaaaaaagaaaaaaaaaaaaaaaaa

SEQ ID NO: 58 - DNA, 190 bp, synthetic construct
  source 1..190: mol_type = other DNA
acaaagttctgtagtgcactgatccataaagtaggaaacactacacgcattattactcacggtacgaaaaaaaaaaaaaaaaaaaaaaaaaaaaaaaaaaaaaaaaaaaaaaaaaaaaaaaaaaaaagatatcaaaaaaaaaaaaaaaaaaagaaaaaaaaaaaaaaaaaaagaaaaaaaaaaaaaaaaa

SEQ ID NO: 59 - DNA, 190 bp, synthetic construct
  source 1..190: mol_type = other DNA
acaaagttctgtagtgcactgacgcattattactcacggtacgatccataaagtaggaaacactacaaaaaaaaaaaaaaaaaaaaaaaaaaaaaaaaaaaaaaaaaaaaaaaaaaaaaaaaaaaaagatatcaaaaaaaaaaaaaaaaaaagaaaaaaaaaaaaaaaaaaagaaaaaaaaaaaaaaaaa

SEQ ID NO: 60-62 - skipped (3 entries)

SEQ ID NO: 63 - DNA, 10 bp, synthetic construct
  source 1..10: mol_type = other DNA
gcatatgact

SEQ ID NO: 64 - DNA, 12 bp, synthetic construct
  source 1..12: mol_type = other DNA
gatatcgtatac

SEQ ID NO: 65 - DNA, 83 bp, synthetic construct
  source 1..83: mol_type = other DNA
tccataaagtaggaaacactacaaaaaaaaaaaaaaaaaaaaaaaaaaaaaaaaaaaaaaaaaaaaaaaaaaaaaaaaaaaaa

SEQ ID NO: 66 - DNA, 83 bp, synthetic construct
  source 1..83: mol_type = other DNA
aaaaaaaaaaaaaaaaaaaaaaaaaaaaaatccataaagtaggaaacactacaaaaaaaaaaaaaaaaaaaaaaaaaaaaaaa

SEQ ID NO: 67 - DNA, 110 bp, synthetic construct
  source 1..110: mol_type = other DNA
aaaaaaaaaaaaaaaaaaaaaaaaaaaaaagcatatgactaaaaaaaaaaaaaaaaaaaaaaaaaaaaaaaaaaaaaaaaaaaaaaaaaaaaaaaaaaaaaaaaaaaaaa

SEQ ID NO: 68 - DNA, 133 bp, synthetic construct
  source 1..133: mol_type = other DNA
tccataaagtaggaaacactacaaaaaaaaaaaaaaaaaaaaaaaaaaaaaaagcatatgactaaaaaaaaaaaaaaaaaaaaaaaaaaaaaaaaaaaaaaaaaaaaaaaaaaaaaaaaaaaaaaaaaaaaaa

SEQ ID NO: 69 - DNA, 133 bp, synthetic construct
  source 1..133: mol_type = other DNA
aaaaaaaaaaaaaaaaaaaaaaaaaaaaaatccataaagtaggaaacactacagcatatgactaaaaaaaaaaaaaaaaaaaaaaaaaaaaaaaaaaaaaaaaaaaaaaaaaaaaaaaaaaaaaaaaaaaaaa

SEQ ID NO: 70 - DNA, 133 bp, synthetic construct
  source 1..133: mol_type = other DNA
aaaaaaaaaaaaaaaaaaaaaaaaaaaaaagcatatgactaaaaaaaaaaaaaaaaaaaatccataaagtaggaaacactacaaaaaaaaaaaaaaaaaaaaaaaaaaaaaaaaaaaaaaaaaaaaaaaaaaa

SEQ ID NO: 71 - DNA, 133 bp, synthetic construct
  source 1..133: mol_type = other DNA
aaaaaaaaaaaaaaaaaaaaaaaaaaaaaagcatatgactaaaaaaaaaaaaaaaaaaaaaaaaaaaaaaaaaaaaaaaaaaaaaaaaaatccataaagtaggaaacactacaaaaaaaaaaaaaaaaaaaaa

SEQ ID NO: 72 - DNA, 37 bp, synthetic construct
  source 1..37: mol_type = other DNA
actcttctggtccccacagactcagagagaacccacc

SEQ ID NO: 73 - DNA, 1653 bp, synthetic construct
  source 1..1653: mol_type = other DNA
atggaagacgccaaaaacattaagaagggcccagcgccattctacccactcgaagacgggaccgccggcgagcagctgcacaaagccatgaagcgctacgccctggtgcccggcaccatcgcctttaccgacgcacatatcgaggtggacattacctacgccgagtacttcgagatgagcgttcggctggcagaagctatgaagcgctatgggctgaatacaaaccatcggatcgtggtgtgcagcgagaatagcttgcagttcttcatgcccgtgttgggtgccctgttcatcggtgtggctgtggccccagctaacgacatctacaacgagcgcgagctgctgaacagcatgggcatcagccagcccaccgtcgtattcgtgagcaagaaagggctgcaaaagatcctcaacgtgcaaaagaagctaccgatcatacaaaagatcatcatcatggatagcaagaccgactaccagggcttccaaagcatgtacaccttcgtgacttcccatttgccacccggcttcaacgagtacgacttcgtgcccgagagcttcgaccgggacaaaaccatcgccctgatcatgaacagtagtggcagtaccggattgcccaagggcgtagccctaccgcaccgcaccgcttgtgtccgattcagtcatgcccgcgaccccatcttcggcaaccagatcatccccgacaccgctatcctcagcgtggtgccatttcaccacggcttcggcatgttcaccacgctgggctacttgatctgcggctttcgggtcgtgctcatgtaccgcttcgaggaggagctattcttgcgcagcttgcaagactataagattcaatctgccctgctggtgcccacactatttagcttcttcgctaagagcactctcatcgacaagtacgacctaagcaacttgcacgagatcgccagcggcggggcgccgctcagcaaggaggtaggtgaggccgtggccaaacgcttccacctaccaggcatccgccagggctacggcctgacagaaacaaccagcgccattctgatcacccccgaaggggacgacaagcctggcgcagtaggcaaggtggtgcccttcttcgaggctaaggtggtggacttggacaccggtaagacactgggtgtgaaccagcgcggcgagctgtgcgtccgtggccccatgatcatgagcggctacgttaacaaccccgaggctacaaacgctctcatcgacaaggacggctggctgcacagcggcgacatcgcctactgggacgaggacgagcacttcttcatcgtggaccggctcaaaagcctgatcaaatacaagggctaccaggtagccccagccgaactggagagcatcctgctgcaacaccccaacatcttcgacgccggggtcgccggcctgcccgacgacgatgccggcgagctgcccgccgcagtcgtcgtgctggaacacggtaaaaccatgaccgagaaggagatcgtggactatgtggccagccaggttacaaccgccaagaagctgcgcggtggtgttgtgttcgtggacgaggtgcctaaaggactgaccggcaagttggacgcccgcaagatccgcgagattctcattaaggccaagaagggcggaaagatcgccgtgtaa